European Patent Application EP 4 450 086 A2, published October 23, 2024. Title: ANTI-IL-17A ANTIBODIES AND THEIR USE IN TREATING AUTOIMMUNE AND INFLAMMATORY DISORDERS. Applicant: Novartis AG. The sequence listing filed with the application follows.

SEQUENCE LISTING (86 sequences)

SEQ ID NO: 1 - protein, 7 aa, Homo sapiens
GFTFSSY

SEQ ID NO: 2 - protein, 6 aa, Homo sapiens
KQDGSE

SEQ ID NO: 3 - protein, 7 aa, Homo sapiens
DRGSLYY

SEQ ID NO: 4 - protein, 7 aa, Homo sapiens
SQGIISA

SEQ ID NO: 5 - skipped

SEQ ID NO: 6 - protein, 6 aa, Homo sapiens
FNSYPL

SEQ ID NO: 7 - protein, 5 aa, Homo sapiens
SYWMS

SEQ ID NO: 8 - protein, 17 aa, Homo sapiens
NIKQDGSEKYYVDSVKG

SEQ ID NO: 9 - protein, 11 aa, Homo sapiens
RPSQGIISALA

SEQ ID NO: 10 - protein, 7 aa, Homo sapiens
DASSLEN

SEQ ID NO: 11 - protein, 9 aa, Homo sapiens
QQFNSYPLT

SEQ ID NO: 12 - protein, 116 aa, Homo sapiens
EVQLVESGGDLVQPGGSLRLSCAASGFTFSSYWMSWVRQAPGKGLEWVANIKQDGSEKYYVDSVKGRFTISRDNAKNSLYLQMNSLRAEDTAVYYCARDRGSLYYWGQGTLVTVSS

SEQ ID NO: 13 - protein, 107 aa, Homo sapiens
AIQLTQSPSSLSASVGDRVTITCRPSQGIISALAWYQQKPGKAPKLLIYDASSLENGVPSRFSGSGSGTDFTLTISSLQPEDFATYYCQQFNSYPLTFGGGTKVEIK

SEQ ID NO: 14 - protein, 446 aa, Homo sapiens
EVQLVESGGDLVQPGGSLRLSCAASGFTFSSYWMSWVRQAPGKGLEWVANIKQDGSEKYYVDSVKGRFTISRDNAKNSLYLQMNSLRAEDTAVYYCARDRGSLYYWGQGTLVTVSSASTKGPSVFPLAPSSKSTSGGTAALGCLVKDYFPEPVTVSWNSGALTSGVHTFPAVLQSSGLYSLSSVVTVPSSSLGTQTYICNVNHKPSNTKVDKRVEPKSCDKTHTCPPCPAPELLGGPSVFLFPPKPKDTLMISRTPEVTCVVVDVSHEDPEVKFNWYVDGVEVHNAKTKPREEQYNSTYRVVSVLTVLHQDWLNGKEYKCKVSNKALPAPIEKTISKAKGQPREPQVYTLPPSREEMTKNQVSLTCLVKGFYPSDIAVEWESNGQPENNYKTTPPVLDSDGSFFLYSKLTVDKSRWQQGNVFSCSVMHEALHNHYTQKSLSLSPGK

SEQ ID NO: 15 - protein, 214 aa, Homo sapiens
AIQLTQSPSSLSASVGDRVTITCRPSQGIISALAWYQQKPGKAPKLLIYDASSLENGVPSRFSGSGSGTDFTLTISSLQPEDFATYYCQQFNSYPLTFGGGTKVEIKRTVAAPSVFIFPPSDEQLKSGTASVVCLLNNFYPREAKVQWKVDNALQSGNSQESVTEQDSKDSTYSLSSTLTLSKADYEKHKVYACEVTHQGLSSPVTKSFNRGEC

SEQ ID NO: 16 - DNA, 348 bp, Homo sapiens
  source 1..348: mol_type = genomic DNA
gaggtgcagctggtcgagtctggcggcgacctggtgcagcctggcggcagcctgagactgagctgcgccgccagcggcttcaccttcagcagctactggatgtcctgggtccgccaggcccctggcaaaggcctcgaatgggtggccaacatcaagcaggacggcagcgagaagtactacgtggacagcgtgaagggccggttcaccatcagccgggacaacgccaagaacagcctgtacctgcagatgaacagcctgcgggccgaggacaccgccgtgtactactgcgccagggaccggggcagcctgtactattggggccagggcaccctggtcaccgtgtccagc

SEQ ID NO: 17 - DNA, 321 bp, Homo sapiens
  source 1..321: mol_type = genomic DNA
gccatccagttgacccagtctccatcctccctgtctgcatctgtgggagacagagtcaccatcacttgccggccaagtcagggcattatcagtgctttagcctggtatcagcagaaaccagggaaagctcctaagctcctgatctatgatgcctccagtttggaaaatggggtcccatcaaggttcagcggcagtggatctgggacagatttcactctcaccatcagcagcctgcagcctgaagattttgcaacttattactgtcaacagtttaatagttaccctctcactttcggcggagggaccaaggtggagatcaaa

SEQ ID NO: 18 - DNA, 1338 bp, Homo sapiens
  source 1..1338: mol_type = genomic DNA
gaggtgcagctggtcgagtctggcggcgacctggtgcagcctggcggcagcctgagactgagctgcgccgccagcggcttcaccttcagcagctactggatgtcctgggtccgccaggcccctggcaaaggcctcgaatgggtggccaacatcaagcaggacggcagcgagaagtactacgtggacagcgtgaagggccggttcaccatcagccgggacaacgccaagaacagcctgtacctgcagatgaacagcctgcgggccgaggacaccgccgtgtactactgcgccagggaccggggcagcctgtactattggggccagggcaccctggtcaccgtgtccagcgctagcaccaagggccccagcgtgttccccctggcccccagcagcaagagcaccagcggcggcacagccgccctgggctgcctggtgaaggactacttccccgagcccgtgaccgtgtcctggaacagcggagccctgacctccggcgtgcacaccttccccgccgtgctgcagagcagcggcctgtacagcctgtccagcgtggtgacagtgcccagcagcagcctgggcacccagacctacatctgcaacgtgaaccacaagcccagcaacaccaaggtggacaagagagtggagcccaagagctgcgacaagacccacacctgccccccctgcccagccccagagctgctgggcggaccctccgtgttcctgttcccccccaagcccaaggacaccctgatgatcagcaggacccccgaggtgacctgcgtggtggtggacgtgagccacgaggacccagaggtgaagttcaactggtacgtggacggcgtggaggtgcacaacgccaagaccaagcccagagaggagcagtacaacagcacctacagggtggtgtccgtgctgaccgtgctgcaccaggactggctgaacggcaaggaatacaagtgcaaggtctccaacaaggccctgccagcccccatcgaaaagaccatcagcaaggccaagggccagccacgggagccccaggtgtacaccctgcccccctcccgggaggagatgaccaagaaccaggtgtccctgacctgtctggtgaagggcttctaccccagcgacatcgccgtggagtgggagagcaacggccagcccgagaacaactacaagaccacccccccagtgctggacagcgacggcagcttcttcctgtacagcaagctgaccgtggacaagtccaggtggcagcagggcaacgtgttcagctgcagcgtgatgcacgaggccctgcacaaccactacacccagaagagcctgagcctgtcccccggcaag

SEQ ID NO: 19 - DNA, 642 bp, Homo sapiens
  source 1..642: mol_type = genomic DNA
gccatccagttgacccagtctccatcctccctgtctgcatctgtgggagacagagtcaccatcacttgccggccaagtcagggcattatcagtgctttagcctggtatcagcagaaaccagggaaagctcctaagctcctgatctatgatgcctccagtttggaaaatggggtcccatcaaggttcagcggcagtggatctgggacagatttcactctcaccatcagcagcctgcagcctgaagattttgcaacttattactgtcaacagtttaatagttaccctctcactttcggcggagggaccaaggtggagatcaaacgtacggtggccgctcccagcgtgttcatcttcccccccagcgacgagcagctgaagagcggcaccgccagcgtggtgtgcctgctgaacaacttctacccccgggaggccaaggtgcagtggaaggtggacaacgccctgcagagcggcaacagccaggagagcgtcaccgagcaggacagcaaggactccacctacagcctgagcagcaccctgaccctgagcaaggccgactacgagaagcataaggtgtacgcctgcgaggtgacccaccagggcctgtccagccccgtgaccaagagcttcaacaggggcgagtgc

SEQ ID NO: 20 - protein, 7 aa, Homo sapiens
SQVIISA

SEQ ID NO: 21 - protein, 6 aa, Homo sapiens
FDSYPL

SEQ ID NO: 22 - protein, 11 aa, Homo sapiens
RPSQVIISALA

SEQ ID NO: 23 - protein, 7 aa, Homo sapiens
DASSLEQ

SEQ ID NO: 24 - protein, 9 aa, Homo sapiens
QQFDSYPLT

SEQ ID NO: 25 - protein, 107 aa, Homo sapiens
AIQLTQSPSSLSASVGDRVTITCRPSQVIISALAWYQQKPGKAPKLLIYDASSLEQGVPSRFSGSVSGTDFTLTISSLQPEDFATYYCQQFDSYPLTFGGGTKVEIK

SEQ ID NO: 26 - protein, 214 aa, Homo sapiens
AIQLTQSPSSLSASVGDRVTITCRPSQVIISALAWYQQKPGKAPKLLIYDASSLEQGVPSRFSGSVSGTDFTLTISSLQPEDFATYYCQQFDSYPLTFGGGTKVEIKRTVAAPSVFIFPPSDEQLKSGTASVVCLLNNFYPREAKVQWKVDNALQSGNSQESVTEQDSKDSTYSLSSTLTLSKADYEKHKVYACEVTHQGLSSPVTKSFNRGEC

SEQ ID NO: 27 - DNA, 321 bp, Homo sapiens
  source 1..321: mol_type = genomic DNA
gccatccagctgacccagagccccagcagcctgagcgccagcgtgggcgacagagtgaccatcacctgtcggcccagccaggtcatcatcagcgccctggcctggtatcagcagaagcctggcaaggcccccaagctgctgatctacgacgccagctccctggaacagggcgtgcccagccggttcagcggcagcgtgtccggcaccgacttcaccctgaccatcagctccctgcagcccgaggacttcgccacctactactgccagcagttcgacagctaccccctgaccttcggcggaggcaccaaggtggaaatcaag

SEQ ID NO: 28 - DNA, 642 bp, Homo sapiens
  source 1..642: mol_type = genomic DNA
gccatccagctgacccagagccccagcagcctgagcgccagcgtgggcgacagagtgaccatcacctgtcggcccagccaggtcatcatcagcgccctggcctggtatcagcagaagcctggcaaggcccccaagctgctgatctacgacgccagctccctggaacagggcgtgcccagccggttcagcggcagcgtgtccggcaccgacttcaccctgaccatcagctccctgcagcccgaggacttcgccacctactactgccagcagttcgacagctaccccctgaccttcggcggaggcaccaaggtggaaatcaagcgtacggtggccgctcccagcgtgttcatcttcccccccagcgacgagcagctgaagagcggcaccgccagcgtggtgtgcctgctgaacaacttctacccccgggaggccaaggtgcagtggaaggtggacaacgccctgcagagcggcaacagccaggagagcgtcaccgagcaggacagcaaggactccacctacagcctgagcagcaccctgaccctgagcaaggccgactacgagaagcataaggtgtacgcctgcgaggtgacccaccagggcctgtccagccccgtgaccaagagcttcaacaggggcgagtgc

SEQ ID NO: 29 - DNA, 348 bp, Homo sapiens
  source 1..348: mol_type = genomic DNA
gaggtgcagctggtggaatcaggaggcgacctggtgcagcctggcggctcactgagactgagctgcgccgctagtggcttcacctttagtagctactggatgagctgggtgcgacaggcccctggcaagggactggagtgggtggccaatattaagcaggacggctcagagaagtactacgtggactcagtgaagggccggttcactattagccgggataacgctaagaatagcctgtacctgcagatgaatagcctgagagccgaggacaccgccgtgtactactgcgctagagatagaggctcactgtactactggggccagggcaccctggtgacagtgtcttct

SEQ ID NO: 30 - DNA, 321 bp, Homo sapiens
  source 1..321: mol_type = genomic DNA
gctattcagctgactcagtcacctagtagcctgagcgctagtgtgggcgatagagtgactatcacctgtagacctagtcaggtgatcattagcgccctggcctggtatcagcagaagcccggcaaggcccctaagctgctgatctacgacgctagtagtctggaacagggcgtgccctctaggtttagcggctcagtgtcaggcaccgacttcaccctgactattagtagcctgcagcccgaggacttcgctacctactactgtcagcagttcgatagctaccccctgaccttcggcggaggcactaaggtggaaatcaag

SEQ ID NO: 31 - DNA, 1338 bp, Homo sapiens
  source 1..1338: mol_type = genomic DNA
gaggtgcagctggtggaatcaggaggcgacctggtgcagcctggcggctcactgagactgagctgcgccgctagtggcttcacctttagtagctactggatgagctgggtgcgacaggcccctggcaagggactggagtgggtggccaatattaagcaggacggctcagagaagtactacgtggactcagtgaagggccggttcactattagccgggataacgctaagaatagcctgtacctgcagatgaatagcctgagagccgaggacaccgccgtgtactactgcgctagagatagaggctcactgtactactggggccagggcaccctggtgacagtgtcttctgctagcaccaagggcccaagtgtctttcccctggcccccagcagcaagtccacaagcggaggcactgcagctctgggttgtctggtgaaggactacttccccgagcccgtgacagtgtcctggaacagcggagccctgacctccggcgtgcacaccttccccgccgtgctgcagagcagcggcctgtacagcctgagcagcgtcgtgactgtgcctagttccagcctgggcacccagacctatatctgcaacgtgaaccacaagcccagcaacaccaaggtggacaagagagtggagcccaagagctgcgacaagacccacacctgccccccctgcccagctccagaactgctgggaggacccagcgtgttcctgttcccccccaagcccaaggacaccctgatgatcagcaggacccccgaggtgacctgcgtggtggtggacgtgtcccacgaggacccagaggtgaagttcaactggtacgtggacggggtggaggtgcacaacgccaagaccaagcccagagaggagcagtacaacagcacctacagggtggtgtccgtcctgacagtgctgcaccaggattggctgaacggcaaagaatacaagtgcaaagtctccaacaaggccctgccagccccaatcgaaaagacaatcagcaaggccaagggccagccacgggagccccaggtgtacaccctgccccccagccgggaggagatgaccaagaaccaggtgtccctgacctgtctggtgaagggcttctaccccagcgatatcgccgtggagtgggagagcaacggccagcccgagaacaactacaagaccacccccccagtgctggacagcgacggcagcttcttcctgtacagcaagctgaccgtggacaagtccaggtggcagcagggcaacgtgttcagctgcagcgtgatgcacgaggccctgcacaaccactacacccagaagtccctgagcctgagccccggcaag

SEQ ID NO: 32 - DNA, 642 bp, Homo sapiens
  source 1..642: mol_type = genomic DNA
gctattcagctgactcagtcacctagtagcctgagcgctagtgtgggcgatagagtgactatcacctgtagacctagtcaggtgatcattagcgccctggcctggtatcagcagaagcccggcaaggcccctaagctgctgatctacgacgctagtagtctggaacagggcgtgccctctaggtttagcggctcagtgtcaggcaccgacttcaccctgactattagtagcctgcagcccgaggacttcgctacctactactgtcagcagttcgatagctaccccctgaccttcggcggaggcactaaggtggaaatcaagcgtacggtggccgctcccagcgtgttcatcttcccccccagcgacgagcagctgaagagcggcaccgccagcgtggtgtgcctgctgaacaacttctacccccgggaggccaaggtgcagtggaaggtggacaacgccctgcagagcggcaacagccaggagagcgtcaccgagcaggacagcaaggactccacctacagcctgagcagcaccctgaccctgagcaaggccgactacgagaagcataaggtgtacgcctgcgaggtgacccaccagggcctgtccagccccgtgaccaagagcttcaacaggggcgagtgc

SEQ ID NO: 33 - protein, 7 aa, Homo sapiens
SQGIYWE

SEQ ID NO: 34 - protein, 11 aa, Homo sapiens
RPSQGIYWELA

SEQ ID NO: 35 - protein, 107 aa, Homo sapiens
AIQLTQSPSSLSASVGDRVTITCRPSQGIYWELAWYQQKPGKAPKLLIYDASSLEQGVPSRFSGSGSGTDFTLTISSLQPEDFATYYCQQFNSYPLTFGGGTKVEIK

SEQ ID NO: 36 - protein, 214 aa, Homo sapiens
AIQLTQSPSSLSASVGDRVTITCRPSQGIYWELAWYQQKPGKAPKLLIYDASSLEQGVPSRFSGSGSGTDFTLTISSLQPEDFATYYCQQFNSYPLTFGGGTKVEIKRTVAAPSVFIFPPSDEQLKSGTASVVCLLNNFYPREAKVQWKVDNALQSGNSQESVTEQDSKDSTYSLSSTLTLSKADYEKHKVYACEVTHQGLSSPVTKSFNRGEC

SEQ ID NO: 37 - DNA, 321 bp, Homo sapiens
  source 1..321: mol_type = genomic DNA
gccatccagctgacccagagccccagcagcctgagcgccagcgtgggcgacagagtgaccatcacctgtcggcccagccagggcatctactgggagctggcctggtatcagcagaagcctggcaaggcccccaagctgctgatctacgacgccagctccctggaacagggcgtgcccagccggttcagcggcagcggatccggcaccgacttcaccctgaccatcagctccctgcagcccgaggacttcgccacctactactgccagcagttcaacagctaccccctgaccttcggcggaggcaccaaggtggaaatcaag

SEQ ID NO: 38 - DNA, 642 bp, Homo sapiens
  source 1..642: mol_type = genomic DNA
gccatccagctgacccagagccccagcagcctgagcgccagcgtgggcgacagagtgaccatcacctgtcggcccagccagggcatctactgggagctggcctggtatcagcagaagcctggcaaggcccccaagctgctgatctacgacgccagctccctggaacagggcgtgcccagccggttcagcggcagcggatccggcaccgacttcaccctgaccatcagctccctgcagcccgaggacttcgccacctactactgccagcagttcaacagctaccccctgaccttcggcggaggcaccaaggtggaaatcaagcgtacggtggccgctcccagcgtgttcatcttcccccccagcgacgagcagctgaagagcggcaccgccagcgtggtgtgcctgctgaacaacttctacccccgggaggccaaggtgcagtggaaggtggacaacgccctgcagagcggcaacagccaggagagcgtcaccgagcaggacagcaaggactccacctacagcctgagcagcaccctgaccctgagcaaggccgactacgagaagcataaggtgtacgcctgcgaggtgacccaccagggcctgtccagccccgtgaccaagagcttcaacaggggcgagtgc

SEQ ID NO: 39 - DNA, 321 bp, Homo sapiens
  source 1..321: mol_type = genomic DNA
gctattcagctgactcagtcacctagtagcctgagcgctagtgtgggcgatagagtgactatcacctgtagacctagccagggaatctactgggagctggcctggtatcagcagaagcccggcaaggcccctaagctgctgatctacgacgctagtagtctggaacagggcgtgccctctaggtttagcggctcaggctcaggcaccgacttcaccctgactattagtagcctgcagcccgaggacttcgctacctactactgtcagcagtttaactcctaccccctgaccttcggcggaggcactaaggtggaaatcaag

SEQ ID NO: 40 - DNA, 642 bp, Homo sapiens
  source 1..642: mol_type = genomic DNA
gctattcagctgactcagtcacctagtagcctgagcgctagtgtgggcgatagagtgactatcacctgtagacctagccagggaatctactgggagctggcctggtatcagcagaagcccggcaaggcccctaagctgctgatctacgacgctagtagtctggaacagggcgtgccctctaggtttagcggctcaggctcaggcaccgacttcaccctgactattagtagcctgcagcccgaggacttcgctacctactactgtcagcagtttaactcctaccccctgaccttcggcggaggcactaaggtggaaatcaagcgtacggtggccgctcccagcgtgttcatcttcccccccagcgacgagcagctgaagagcggcaccgccagcgtggtgtgcctgctgaacaacttctacccccgggaggccaaggtgcagtggaaggtggacaacgccctgcagagcggcaacagccaggagagcgtcaccgagcaggacagcaaggactccacctacagcctgagcagcaccctgaccctgagcaaggccgactacgagaagcataaggtgtacgcctgcgaggtgacccaccagggcctgtccagccccgtgaccaagagcttcaacaggggcgagtgc

SEQ ID NO: 41 - protein, 7 aa, Homo sapiens
SQGINWE

SEQ ID NO: 42 - protein, 11 aa, Homo sapiens
RPSQGINWELA

SEQ ID NO: 43 - protein, 107 aa, Homo sapiens
AIQLTQSPSSLSASVGDRVTITCRPSQGINWELAWYQQKPGKAPKLLIYDASSLEQGVPSRFSGSGSGTDFTLTISSLQPEDFATYYCQQFNSYPLTFGGGTKVEIK

SEQ ID NO: 44 - protein, 214 aa, Homo sapiens
AIQLTQSPSSLSASVGDRVTITCRPSQGINWELAWYQQKPGKAPKLLIYDASSLEQGVPSRFSGSGSGTDFTLTISSLQPEDFATYYCQQFNSYPLTFGGGTKVEIKRTVAAPSVFIFPPSDEQLKSGTASVVCLLNNFYPREAKVQWKVDNALQSGNSQESVTEQDSKDSTYSLSSTLTLSKADYEKHKVYACEVTHQGLSSPVTKSFNRGEC

SEQ ID NO: 45 - DNA, 321 bp, Homo sapiens
  source 1..321: mol_type = genomic DNA
gccatccagctgacccagagccccagcagcctgagcgccagcgtgggcgacagagtgaccatcacctgtcggcccagccagggcatcaactgggagctggcctggtatcagcagaagcctggcaaggcccccaagctgctgatctacgacgccagctccctggaacagggcgtgcccagccggttcagcggcagcggatccggcaccgacttcaccctgaccatcagctccctgcagcccgaggacttcgccacctactactgccagcagttcaacagctaccccctgaccttcggcggaggcaccaaggtggaaatcaag

SEQ ID NO: 46 - DNA, 642 bp, Homo sapiens
  source 1..642: mol_type = genomic DNA
gccatccagctgacccagagccccagcagcctgagcgccagcgtgggcgacagagtgaccatcacctgtcggcccagccagggcatcaactgggagctggcctggtatcagcagaagcctggcaaggcccccaagctgctgatctacgacgccagctccctggaacagggcgtgcccagccggttcagcggcagcggatccggcaccgacttcaccctgaccatcagctccctgcagcccgaggacttcgccacctactactgccagcagttcaacagctaccccctgaccttcggcggaggcaccaaggtggaaatcaagcgtacggtggccgctcccagcgtgttcatcttcccccccagcgacgagcagctgaagagcggcaccgccagcgtggtgtgcctgctgaacaacttctacccccgggaggccaaggtgcagtggaaggtggacaacgccctgcagagcggcaacagccaggagagcgtcaccgagcaggacagcaaggactccacctacagcctgagcagcaccctgaccctgagcaaggccgactacgagaagcataaggtgtacgcctgcgaggtgacccaccagggcctgtccagccccgtgaccaagagcttcaacaggggcgagtgc

SEQ ID NO: 47 - DNA, 321 bp, Homo sapiens
  source 1..321: mol_type = genomic DNA
gctattcagctgactcagtcacctagtagcctgagcgctagtgtgggcgatagagtgactatcacctgtagacctagtcaggggattaactgggagctggcctggtatcagcagaagcccggcaaggcccctaagctgctgatctacgacgctagtagtctggaacagggcgtgccctctaggtttagcggctcaggctcaggcaccgacttcaccctgactattagtagcctgcagcccgaggacttcgctacctactactgtcagcagtttaactcctaccccctgaccttcggcggaggcactaaggtggaaatcaag

SEQ ID NO: 48 - DNA, 642 bp, Homo sapiens
  source 1..642: mol_type = genomic DNA
gctattcagctgactcagtcacctagtagcctgagcgctagtgtgggcgatagagtgactatcacctgtagacctagtcaggggattaactgggagctggcctggtatcagcagaagcccggcaaggcccctaagctgctgatctacgacgctagtagtctggaacagggcgtgccctctaggtttagcggctcaggctcaggcaccgacttcaccctgactattagtagcctgcagcccgaggacttcgctacctactactgtcagcagtttaactcctaccccctgaccttcggcggaggcactaaggtggaaatcaagcgtacggtggccgctcccagcgtgttcatcttcccccccagcgacgagcagctgaagagcggcaccgccagcgtggtgtgcctgctgaacaacttctacccccgggaggccaaggtgcagtggaaggtggacaacgccctgcagagcggcaacagccaggagagcgtcaccgagcaggacagcaaggactccacctacagcctgagcagcaccctgaccctgagcaaggccgactacgagaagcataaggtgtacgcctgcgaggtgacccaccagggcctgtccagccccgtgaccaagagcttcaacaggggcgagtgc

SEQ ID NO: 49 - DNA, 348 bp, Homo sapiens
  source 1..348: mol_type = genomic DNA
gaggtgcagctggtggaatctggcggcgacctggtgcagcctggcggctctctgagactgtcttgcgccgcctccggcttcaccttctccagctactggatgtcctgggtgcgacaggcccctggcaagggactggaatgggtggccaacatcaagcaggacggctccgagaagtactacgtggactccgtgaagggccggttcaccatctcccgggacaacgccaagaactccctgtacctgcagatgaactccctgcgggccgaggacaccgccgtgtactactgcgccagggaccggggctccctgtactattggggccagggcaccctggtgacagtgtcctcc

SEQ ID NO: 50 - DNA, 321 bp, Homo sapiens
  source 1..321: mol_type = genomic DNA
gccatccagctgacccagtccccctccagcctgtctgcctccgtgggcgacagagtgaccatcacctgtcggccctcccagggcatcaactgggaactggcctggtatcagcagaagcccggcaaggcccccaagctgctgatctacgacgccagctccctggaacagggcgtgccctccagattctccggctctggctccggcaccgacttcaccctgaccatctccagcctgcagcccgaggacttcgccacctactactgccagcagttcaactcctaccccctgaccttcggcggaggcaccaaggtggaaatcaag

SEQ ID NO: 51 - DNA, 1338 bp, Homo sapiens
  source 1..1338: mol_type = genomic DNA
gaggtgcagctggtggaatctggcggcgacctggtgcagcctggcggctctctgagactgtcttgcgccgcctccggcttcaccttctccagctactggatgtcctgggtgcgacaggcccctggcaagggactggaatgggtggccaacatcaagcaggacggctccgagaagtactacgtggactccgtgaagggccggttcaccatctcccgggacaacgccaagaactccctgtacctgcagatgaactccctgcgggccgaggacaccgccgtgtactactgcgccagggaccggggctccctgtactattggggccagggcaccctggtgacagtgtcctccgcctccaccaagggcccaagcgtgttccccctggcccccagcagcaagagcaccagcggcggcacagccgccctgggctgcctggtgaaggactacttccccgagcccgtgaccgtgtcctggaacagcggagccctgacctccggcgtgcacaccttccccgccgtgctgcagagcagcggcctgtacagcctgagcagcgtggtgaccgtgcccagcagcagcctgggcacccagacctacatctgtaacgtgaaccacaagcccagcaacaccaaggtggacaagagagtggagcccaagagctgtgacaagacccacacctgccccccctgcccagcccccgagctgctgggcggacccagcgtgttcctgttcccccccaagcccaaggacaccctgatgatcagcagaacccccgaggtgacctgtgtggtggtggacgtgtcccacgaggacccagaggtgaagttcaactggtacgtggacggcgtggaggtgcacaacgccaagaccaagcccagagaggagcagtacaacagcacctacagggtggtgtccgtgctgaccgtgctgcaccaggactggctgaacggcaaggagtacaagtgtaaggtgtccaacaaggccctgccagccccaatcgaaaagaccatcagcaaggccaagggccagccaagagagccccaggtgtacaccctgccacccagcagggaggagatgaccaagaaccaggtgtccctgacctgtctggtgaagggcttctacccaagcgacatcgccgtggagtgggagagcaacggccagcccgagaacaactacaagaccacccccccagtgctggacagcgacggcagcttcttcctgtacagcaagctgaccgtggacaagagcagatggcagcagggcaacgtgttcagctgctccgtgatgcacgaggccctgcacaaccactacacccagaagagcctgagcctgtccccaggcaag

SEQ ID NO: 52 - DNA, 642 bp, Homo sapiens
  source 1..642: mol_type = genomic DNA
gccatccagctgacccagtccccctccagcctgtctgcctccgtgggcgacagagtgaccatcacctgtcggccctcccagggcatcaactgggaactggcctggtatcagcagaagcccggcaaggcccccaagctgctgatctacgacgccagctccctggaacagggcgtgccctccagattctccggctctggctccggcaccgacttcaccctgaccatctccagcctgcagcccgaggacttcgccacctactactgccagcagttcaactcctaccccctgaccttcggcggaggcaccaaggtggaaatcaagcgtacggtggccgctcccagcgtgttcatcttccccccaagcgacgagcagctgaagagcggcaccgccagcgtggtgtgtctgctgaacaacttctaccccagggaggccaaggtgcagtggaaggtggacaacgccctgcagagcggcaacagccaggagagcgtcaccgagcaggacagcaaggactccacctacagcctgagcagcaccctgaccctgagcaaggccgactacgagaagcacaaggtgtacgcctgtgaggtgacccaccagggcctgtccagccccgtgaccaagagcttcaacaggggcgagtgc

SEQ ID NO: 53 - protein, 107 aa, Homo sapiens
AIQLTQSPSSLSASVGDRVTITCRPSQGINWELAWYQQKPGKAPKLLIYDASSLENGVPSRFSGSGSGTDFTLTISSLQPEDFATYYCQQFNSYPLTFGGGTKVEIK

SEQ ID NO: 54 - protein, 214 aa, Homo sapiens
AIQLTQSPSSLSASVGDRVTITCRPSQGINWELAWYQQKPGKAPKLLIYDASSLENGVPSRFSGSGSGTDFTLTISSLQPEDFATYYCQQFNSYPLTFGGGTKVEIKRTVAAPSVFIFPPSDEQLKSGTASVVCLLNNFYPREAKVQWKVDNALQSGNSQESVTEQDSKDSTYSLSSTLTLSKADYEKHKVYACEVTHQGLSSPVTKSFNRGEC

SEQ ID NO: 55 - DNA, 321 bp, Homo sapiens
  source 1..321: mol_type = genomic DNA
gccatccagctgacccagagccccagcagcctgagcgccagcgtgggcgacagagtgaccatcacctgtcggcccagccagggcatcaactgggagctggcctggtatcagcagaagcctggcaaggcccccaagctgctgatctacgacgccagctccctggaaaacggcgtgcccagccggttcagcggcagcggatccggcaccgacttcaccctgaccatcagctccctgcagcccgaggacttcgccacctactactgccagcagttcaacagctaccccctgaccttcggcggaggcaccaaggtggaaatcaag

SEQ ID NO: 56 - DNA, 642 bp, Homo sapiens
  source 1..642: mol_type = genomic DNA
gccatccagctgacccagagccccagcagcctgagcgccagcgtgggcgacagagtgaccatcacctgtcggcccagccagggcatcaactgggagctggcctggtatcagcagaagcctggcaaggcccccaagctgctgatctacgacgccagctccctggaaaacggcgtgcccagccggttcagcggcagcggatccggcaccgacttcaccctgaccatcagctccctgcagcccgaggacttcgccacctactactgccagcagttcaacagctaccccctgaccttcggcggaggcaccaaggtggaaatcaagcgtacggtggccgctcccagcgtgttcatcttcccccccagcgacgagcagctgaagagcggcaccgccagcgtggtgtgcctgctgaacaacttctacccccgggaggccaaggtgcagtggaaggtggacaacgccctgcagagcggcaacagccaggagagcgtcaccgagcaggacagcaaggactccacctacagcctgagcagcaccctgaccctgagcaaggccgactacgagaagcataaggtgtacgcctgcgaggtgacccaccagggcctgtccagccccgtgaccaagagcttcaacaggggcgagtgc

SEQ ID NO: 57 - DNA, 321 bp, Homo sapiens
  source 1..321: mol_type = genomic DNA
gctattcagctgactcagtcacctagtagcctgagcgctagtgtgggcgatagagtgactatcacctgtagacctagtcaggggattaactgggagctggcctggtatcagcagaagcccggcaaggcccctaagctgctgatctacgacgctagtagtctggaaaacggcgtgccctctaggtttagcggctcaggctcaggcaccgacttcaccctgactattagtagcctgcagcccgaggacttcgctacctactactgtcagcagtttaactcctaccccctgaccttcggcggaggcactaaggtggaaatcaag

SEQ ID NO: 58 - DNA, 642 bp, Homo sapiens
  source 1..642: mol_type = genomic DNA
gctattcagctgactcagtcacctagtagcctgagcgctagtgtgggcgatagagtgactatcacctgtagacctagtcaggggattaactgggagctggcctggtatcagcagaagcccggcaaggcccctaagctgctgatctacgacgctagtagtctggaaaacggcgtgccctctaggtttagcggctcaggctcaggcaccgacttcaccctgactattagtagcctgcagcccgaggacttcgctacctactactgtcagcagtttaactcctaccccctgaccttcggcggaggcactaaggtggaaatcaagcgtacggtggccgctcccagcgtgttcatcttcccccccagcgacgagcagctgaagagcggcaccgccagcgtggtgtgcctgctgaacaacttctacccccgggaggccaaggtgcagtggaaggtggacaacgccctgcagagcggcaacagccaggagagcgtcaccgagcaggacagcaaggactccacctacagcctgagcagcaccctgaccctgagcaaggccgactacgagaagcataaggtgtacgcctgcgaggtgacccaccagggcctgtccagccccgtgaccaagagcttcaacaggggcgagtgc

SEQ ID NO: 59 - protein, 19 aa, synthetic construct
  REGION 1..19: note = Heavy chain leader sequence
MEFGLSWVFLVAILEGVHC

SEQ ID NO: 60 - protein, 22 aa, synthetic construct
  REGION 1..22: note = Light chain leader sequence
MDMRVPAQLLGLLLLWLPGARC

SEQ ID NO: 61 - DNA, 57 bp, synthetic construct
  misc_feature 1..57: note = Coding sequence for heavy chain leader sequence
  source 1..57: mol_type = other DNA
atggaattcggcctgagctgggtgttcctggtcgcgattctggaaggcgtgcactgc

SEQ ID NO: 62 - DNA, 66 bp, synthetic construct
  misc_feature 1..66: note = Coding sequence for light chain leader sequence
  source 1..66: mol_type = other DNA
atggacatgagggtccccgctcagctcctggggcttctgctgctctggctcccaggcgccagatgt

SEQ ID NO: 63 - protein, 19 aa, synthetic construct
  REGION 1..19: note = Alternative heavy chain leader sequence
MAWVWTLPFLMAAAQSVQA

SEQ ID NO: 64 - protein, 20 aa, synthetic construct
  REGION 1..20: note = Alternative light chain leader sequence
MSVLTQVLALLLLWLTGTRC

SEQ ID NO: 65 - DNA, 57 bp, synthetic construct
  misc_feature 1..57: note = Coding sequence for alternative heavy chain leader sequence
  source 1..57: mol_type = other DNA
atggcctgggtgtggaccctgcccttcctgatggccgctgctcagtcagtgcaggcc

SEQ ID NO: 66 - DNA, 60 bp, synthetic construct
  misc_feature 1..60: note = Coding sequence for alternative light chain leader sequence
  source 1..60: mol_type = other DNA
atgagcgtgctgactcaggtgctggccctgctgctgctgtggctgaccggcacccgctgc

SEQ ID NO: 67 - protein, 19 aa, synthetic construct
  REGION 1..19: note = Second alternative heavy chain leader sequence
MEWSWVFLFFLSVTTGVHS

SEQ ID NO: 68 - protein, 20 aa, synthetic construct
  REGION 1..20: note = Second alternative light chain leader sequence
MSVPTQVLGLLLLWLTDARC

SEQ ID NO: 69 - DNA, 57 bp, synthetic construct
  misc_feature 1..57: note = Coding sequence for second alternative heavy chain leader sequence
  source 1..57: mol_type = other DNA
atggaatggtcctgggtgttcctgttcttcctgtccgtgaccacaggcgtgcactcc

SEQ ID NO: 70 - DNA, 60 bp, synthetic construct
  misc_feature 1..60: note = Coding sequence for second alternative light chain leader sequence
  source 1..60: mol_type = other DNA
atgtccgtgcccacacaggtgctgggcctgctgctgctgtggctgaccgacgccagatgc

SEQ ID NO: 71 - skipped

SEQ ID NO: 72 - protein, 6 aa, Homo sapiens
  SITE 2: note = Xaa - Variable
FXSYPL

SEQ ID NO: 73 - protein, 11 aa, Homo sapiens
  SITE 5: note = Xaa - Variable
  REGION 7..9: note = Xaa - Variable
RPSQXIXXXLA

SEQ ID NO: 74 - protein, 7 aa, Homo sapiens
  SITE 7: note = Xaa - Variable
DASSLEX

SEQ ID NO: 75 - protein, 9 aa, Homo sapiens
  SITE 4: note = Xaa - Variable
QQFXSYPLT

SEQ ID NO: 76 - protein, 136 aa, Homo sapiens
GITIPRNPGCPNSEDKNFPRTVMVNLNIHNRNTNTNPKRSSDYYNRSTSPWNLHRNEDPERYPSVIWEAKCRHLGCINADGNVDYHMNSVPIQQEILVLRREPPHCPNSFRLEKILVSVGCTCVTPIVHHVAEFRH

SEQ ID NO: 77 - protein, 134 aa, Homo sapiens
MRKIPKVGHTFFQKPESCPPVPGGSMKLDIGIINENQRVSMSRNIESRSTSPWNYTVTWDPNRYPSEVVQAQCRNLGCINAQGKEDISMNSVPIQQETLVVRRKHQGCSVSFQLEKVLVTVGCTCVTPVIHHVQ

SEQ ID NO: 78 - protein, 138 aa, Homo sapiens
GPIVKAGITIPRNPGCPNSEDKNFPRTVMVNLNIHNRNTNTNPKRSSDYYNRSTSPWNLHRNEDPERYPSVIWEAKCRHLGCINADGNVDYHMNSVPIQQEILVLRREPPHCPNSFRLEKILVSVGCTCVTPIVHHVA

SEQ ID NO: 79 - protein, 132 aa, Macaca fascicularis
GIAIPRNSGCPNSEDKNFPRTVMVNLNIHNRNTSTNPKRSSDYYNRSTSPWNLHRNEDPERYPSVIWEAKCRHLGCVKADGNVDYHMNSVPIQQEILVLRREPRHCPNSFRLEKILVSVGCTCVTPIVHHVA

SEQ ID NO: 80 - protein, 134 aa, Macaca fascicularis
MRKIPKVGHTFFQKPESCPPVPEGSMKLDTGIINENQRVSMSRNIESRSTSPWNYTVTWDPNRYPSEVVQAQCKHLGCINAQGKEDISMNSVPIQQETLVLRRKHQGCSVSFQLEKVLVTVGCTCVTPVVHHVQ

SEQ ID NO: 81 - protein, 132 aa, Macaca mulatta
GIAIPRNSGCPNSEDKNFPRTVMVNLNIHNRNTSTSPKRSSDYYNRSTSPWNLHRNEDPERYPSVIWEAKCRHLGCVKADGNVDYHMNSVPIQQEILVLRREPRHCPNSFRLEKILVSVGCTCVTPIVHHVA

SEQ ID NO: 82 - protein, 127 aa, Callithrix jacchus
SPQNPGCPNAEDKNFPRTVMVNLNIRNRNTNSKRASDYYNRSSSPWNLHRNEDPERYPSVIWEAKCRHLGCVDADGNVDYHMNSVPIQQEILVLRREPRHCTNSFRLEKMLVSVGCTCVTPIVHHVA

SEQ ID NO: 83 - protein, 134 aa, Mus musculus
MAAIIPQSSACPNTEAKDFLQNVKVNLKVFNSLGAKVSSRRPSDYLNRSTSPWTLHRNEDPDRYPSVIWEAQCRHQRCVNAEGKLDHHMNSVLIQQEILVLKREPESCPFTFRVEKMLVGVGCTCVASIVRQAA

SEQ ID NO: 84 - protein, 141 aa, Mus musculus
APEPEFRHRKNPKAGVPALQKAGNCPPLEDNTVRVDIRIFNQNQGISVPREFQNRSSSPWDYNITRDPHRFPSEIAEAQCRHSGCINAQGQEDSTMNSVAIQQEILVLRREPQGCSNSFRLEKMLLKVGCTCVKPIVHQAA

SEQ ID NO: 85 - protein, 134 aa, Rattus norvegicus
MAVLIPQSSVCPNAEANNFLQNVKVNLKVINSLSSKASSRRPSDYLNRSTSPWTLSRNEDPDRYPSVIWEAQCRHQRCVNAEGKLDHHMNSVLIQQEILVLKREPEKCPFTFRVEKMLVGVGCTCVSSIVRHAS

SEQ ID NO: 86 - protein, 295 aa, Homo sapiens
NCTVKNSTCLDDSWIHPRNLTPSSPKDLQIQLHFAHTQQGDLFPVAHIEWTLQTDASILYLEGAELSVLQLNTNERLCVRFEFLSKLRHHHRRWRFTFSHFVVDPDQEYEVTVHHLPKPIPDGDPNHQSKNFLVPDCEHARMKVTTPCMSSGSLWDPNITVETLEAHQLRVSFTLWNESTHYQILLTSFPHMENHSCFEHMHHIPAPRPEEFHQRSNVTLTLRNLKGCCRHQVQIQPFFSSCLNDCLRHSATVSCPEMPDTPEPIPDYMPLWEFRHDSGGGLNDIFEAQKIEWHE